European Patent Application EP 4 428 159 A1, published September 11, 2024. Title: MELANOMA TARGETING HUMAN ANTIBODIES AND THERAPEUTIC USES THEREOF. Applicant: Istituto Romagnolo per lo Studio dei Tumori "Dino Amadori" - IRST S.r.l. Application EP. The sequence listing filed with the application follows.

SEQUENCE LISTING (144 sequences)

SEQ ID NO: 1 - protein, 5 aa, synthetic construct
TFTFS

SEQ ID NO: 2 - protein, 17 aa, synthetic construct
RIIPSLGVADYADKFQG

SEQ ID NO: 3 - protein, 15 aa, synthetic construct
NGGYNYGSYYYYMDV

SEQ ID NO: 4 - protein, 5 aa, synthetic construct
DYDIH

SEQ ID NO: 5 - protein, 17 aa, synthetic construct
WINPNTGATGFAQKFQG

SEQ ID NO: 6 - protein, 13 aa, synthetic construct
VCCRSTRSRNLDY

SEQ ID NO: 7 - protein, 15 aa, synthetic construct
DASSGSYAGRAHFDY

SEQ ID NO: 8 - protein, 5 aa, synthetic construct
TSWLT

SEQ ID NO: 9 - protein, 17 aa, synthetic construct
FIHPDGRITYYADSVRG

SEQ ID NO: 10 - protein, 11 aa, synthetic construct
HRRAGAHFFDY

SEQ ID NO: 11 - protein, 12 aa, synthetic construct
RASQSVSSSYLA

SEQ ID NO: 12 - protein, 7 aa, synthetic construct
GASSRAA

SEQ ID NO: 13 - protein, 9 aa, synthetic construct
QQTPLGGWT

SEQ ID NO: 14 - protein, 30 aa, synthetic construct
QVLLAQSGSEVKNPGSSVRVSCKLSGGTFT

SEQ ID NO: 15 - protein, 14 aa, synthetic construct
WLRQAPGQGLEWMG

SEQ ID NO: 16 - protein, 32 aa, synthetic construct
RVTITADKSTSTAYMKVSSLRSEDTAQYYCAK

SEQ ID NO: 17 - protein, 11 aa, synthetic construct
WGQGTTVIVSS

SEQ ID NO: 18 - protein, 30 aa, synthetic construct
QVRLVQSGAEVKKPGASVKVSCQPSGYYFT

SEQ ID NO: 19 - protein, 14 aa, synthetic construct
WVRQAPGQGLEWMG

SEQ ID NO: 20 - protein, 32 aa, synthetic construct
RVTMTRDTSIKIGFMQLFSLTSDDTAVYYCAR

SEQ ID NO: 21 - protein, 11 aa, synthetic construct
WGQGTLVTVSS

SEQ ID NO: 22 - protein, 30 aa, synthetic construct; identical to SEQ ID NO: 14

SEQ ID NO: 23 - protein, 32 aa, synthetic construct
RVTITADKSTSTAYMKVSSLRSEDTAQYYCAR

SEQ ID NO: 24 - protein, 30 aa, synthetic construct
EVQLVESGGGLVQPGGSLRLSCAGSKFPFS

SEQ ID NO: 25 - protein, 14 aa, synthetic construct
WVRQAPGKGLEWLA

SEQ ID NO: 26 - protein, 32 aa, synthetic construct
RFTISRDNARNSVYLQMSSLRDDDTALYYCAR

SEQ ID NO: 27 - protein, 11 aa, synthetic construct
WGQGTMVTVSS

SEQ ID NO: 28 - protein, 25 aa, synthetic construct
QVLLAQSGSEVKNPGSSVRVSCKLS

SEQ ID NO: 29 - protein, 29 aa, synthetic construct
QVLLAQSGSEVKNPGSSVRVSCKLSGGTF

SEQ ID NO: 30 - protein, 7 aa, synthetic construct
GGTFTTF

SEQ ID NO: 31 - protein, 10 aa, synthetic construct
GGTFTTFTFS

SEQ ID NO: 32 - protein, 6 aa, synthetic construct
TTFTFS

SEQ ID NO: 33 - protein, 8 aa, synthetic construct
GGTFTTFT

SEQ ID NO: 34 - protein, 19 aa, synthetic construct
TFSWLRQAPGQGLEWMGRI

SEQ ID NO: 35 - protein, 11 aa, synthetic construct
WLRQAPGQGLE

SEQ ID NO: 36 - protein, 17 aa, synthetic construct
FSWLRQAPGQGLEWMGR

SEQ ID NO: 37 - protein, 6 aa, synthetic construct
IPSLGV

SEQ ID NO: 38 - protein, 10 aa, synthetic construct
RIIPSLGVAD

SEQ ID NO: 39 - protein, 13 aa, synthetic construct
WMGRIIPSLGVAD

SEQ ID NO: 40 - protein, 8 aa, synthetic construct
IIPSLGVA

SEQ ID NO: 41 - protein, 41 aa, synthetic construct
ADYADKFQGRVTITADKSTSTAYMKVSSLRSEDTAQYYCAK

SEQ ID NO: 42 - protein, 39 aa, synthetic construct
YADKFQGRVTITADKSTSTAYMKVSSLRSEDTAQYYCAK

SEQ ID NO: 43 - protein, 37 aa, synthetic construct
YADKFQGRVTITADKSTSTAYMKVSSLRSEDTAQYYC

SEQ ID NO: 44 - protein, 38 aa, synthetic construct
DYADKFQGRVTITADKSTSTAYMKVSSLRSEDTAQYYC

SEQ ID NO: 45 - protein, 16 aa, synthetic construct
AKNGGYNYGSYYYYMD

SEQ ID NO: 46 - protein, 17 aa, synthetic construct
AKNGGYNYGSYYYYMDV

SEQ ID NO: 47 - protein, 12 aa, synthetic construct
VWGQGTTVIVSS

SEQ ID NO: 48 - protein, 25 aa, synthetic construct
QVRLVQSGAEVKKPGASVKVSCQPS

SEQ ID NO: 49 - protein, 29 aa, synthetic construct
QVRLVQSGAEVKKPGASVKVSCQPSGYYF

SEQ ID NO: 50 - protein, 7 aa, synthetic construct
GYYFTDY

SEQ ID NO: 51 - protein, 10 aa, synthetic construct
GYYFTDYDIH

SEQ ID NO: 52 - protein, 6 aa, synthetic construct
TDYDIH

SEQ ID NO: 53 - protein, 8 aa, synthetic construct
GYYFTDYD

SEQ ID NO: 54 - protein, 19 aa, synthetic construct
DIHWVRQAPGQGLEWMGWI

SEQ ID NO: 55 - protein, 11 aa, synthetic construct
WVRQAPGQGLE

SEQ ID NO: 56 - protein, 17 aa, synthetic construct
IHWVRQAPGQGLEWMGW

SEQ ID NO: 57 - protein, 6 aa, synthetic construct
NPNTGA

SEQ ID NO: 58 - protein, 10 aa, synthetic construct
WINPNTGATG

SEQ ID NO: 59 - protein, 13 aa, synthetic construct
WMGWINPNTGATG

SEQ ID NO: 60 - protein, 8 aa, synthetic construct
INPNTGAT

SEQ ID NO: 61 - protein, 41 aa, synthetic construct
TGFAQKFQGRVTMTRDTSIKIGFMQLFSLTSDDTAVYYCAR

SEQ ID NO: 62 - protein, 39 aa, synthetic construct
FAQKFQGRVTMTRDTSIKIGFMQLFSLTSDDTAVYYCAR

SEQ ID NO: 63 - protein, 37 aa, synthetic construct
FAQKFQGRVTMTRDTSIKIGFMQLFSLTSDDTAVYYC

SEQ ID NO: 64 - protein, 38 aa, synthetic construct
GFAQKFQGRVTMTRDTSIKIGFMQLFSLTSDDTAVYYC

SEQ ID NO: 65 - protein, 14 aa, synthetic construct
ARVCCRSTRSRNLD

SEQ ID NO: 66 - protein, 15 aa, synthetic construct
ARVCCRSTRSRNLDY

SEQ ID NO: 67 - protein, 12 aa, synthetic construct
YWGQGTLVTVSS

SEQ ID NO: 68 - protein, 25 aa, synthetic construct
QVLLAQSGSEVKNPGSSVRVSCKLS

SEQ ID NO: 69 - protein, 29 aa, synthetic construct
QVLLAQSGSEVKNPGSSVRVSCKLSGGTF

SEQ ID NO: 70 - protein, 7 aa, synthetic construct
GGTFTTF

SEQ ID NO: 71 - protein, 10 aa, synthetic construct
GGTFTTFTFS

SEQ ID NO: 72 - protein, 6 aa, synthetic construct
TTFTFS

SEQ ID NO: 73 - protein, 8 aa, synthetic construct
GGTFTTFT

SEQ ID NO: 74 - protein, 19 aa, synthetic construct
TFSWLRQAPGQGLEWMGRI

SEQ ID NO: 75 - protein, 11 aa, synthetic construct
WLRQAPGQGLE

SEQ ID NO: 76 - protein, 17 aa, synthetic construct
FSWLRQAPGQGLEWMGR

SEQ ID NO: 77 - protein, 6 aa, synthetic construct
IPSLGV

SEQ ID NO: 78 - protein, 10 aa, synthetic construct
RIIPSLGVAD

SEQ ID NO: 79 - protein, 13 aa, synthetic construct
WMGRIIPSLGVAD

SEQ ID NO: 80 - protein, 8 aa, synthetic construct
IIPSLGVA

SEQ ID NO: 81 - protein, 41 aa, synthetic construct
ADYADKFQGRVTITADKSTSTAYMKVSSLRSEDTAQYYCAR

SEQ ID NO: 82 - protein, 39 aa, synthetic construct
YADKFQGRVTITADKSTSTAYMKVSSLRSEDTAQYYCAR

SEQ ID NO: 83 - protein, 37 aa, synthetic construct; identical to SEQ ID NO: 43

SEQ ID NO: 84 - protein, 38 aa, synthetic construct; identical to SEQ ID NO: 44

SEQ ID NO: 85 - protein, 16 aa, synthetic construct
ARDASSGSYAGRAHFD

SEQ ID NO: 86 - protein, 17 aa, synthetic construct
ARDASSGSYAGRAHFDY

SEQ ID NO: 87 - protein, 12 aa, synthetic construct
YWGQGTTVIVSS

SEQ ID NO: 88 - protein, 25 aa, synthetic construct
EVQLVESGGGLVQPGGSLRLSCAGS

SEQ ID NO: 89 - protein, 29 aa, synthetic construct
EVQLVESGGGLVQPGGSLRLSCAGSKFPF

SEQ ID NO: 90 - protein, 7 aa, synthetic construct
KFPFSTS

SEQ ID NO: 91 - protein, 10 aa, synthetic construct
KFPFSTSWLT

SEQ ID NO: 92 - protein, 6 aa, synthetic construct
STSWLT

SEQ ID NO: 93 - protein, 8 aa, synthetic construct
KFPFSTSW

SEQ ID NO: 94 - protein, 19 aa, synthetic construct
WLTWVRQAPGKGLEWLAFI

SEQ ID NO: 95 - protein, 11 aa, synthetic construct
WVRQAPGKGLE

SEQ ID NO: 96 - protein, 17 aa, synthetic construct
LTWVRQAPGKGLEWLAF

SEQ ID NO: 97 - protein, 6 aa, synthetic construct
HPDGRI

SEQ ID NO: 98 - protein, 10 aa, synthetic construct
FIHPDGRITY

SEQ ID NO: 99 - protein, 13 aa, synthetic construct
WLAFIHPDGRITY

SEQ ID NO: 100 - protein, 8 aa, synthetic construct
IHPDGRIT

SEQ ID NO: 101 - protein, 41 aa, synthetic construct
TYYADSVRGRFTISRDNARNSVYLQMSSLRDDDTALYYCAR

SEQ ID NO: 102 - protein, 39 aa, synthetic construct
YADSVRGRFTISRDNARNSVYLQMSSLRDDDTALYYCAR

SEQ ID NO: 103 - protein, 37 aa, synthetic construct
YADSVRGRFTISRDNARNSVYLQMSSLRDDDTALYYC

SEQ ID NO: 104 - protein, 38 aa, synthetic construct
YYADSVRGRFTISRDNARNSVYLQMSSLRDDDTALYYC

SEQ ID NO: 105 - protein, 12 aa, synthetic construct
ARHRRAGAHFFD

SEQ ID NO: 106 - protein, 13 aa, synthetic construct
ARHRRAGAHFFDY

SEQ ID NO: 107 - protein, 12 aa, synthetic construct
YWGQGTMVTVSS

SEQ ID NO: 108 - protein, 23 aa, synthetic construct
EIVLTQSPGTLSLSPGERATLSC

SEQ ID NO: 109 - protein, 15 aa, synthetic construct
WYQQKPGQAPRLLIY

SEQ ID NO: 110 - protein, 32 aa, synthetic construct
GIPDRFSGSGSGTDFTLTISRLEPEDFAVYYC

SEQ ID NO: 111 - protein, 10 aa, synthetic construct
FGQGTKVEIK

SEQ ID NO: 112 - protein, 29 aa, synthetic construct
EIVLTQSPGTLSLSPGERATLSCRASQSV

SEQ ID NO: 113 - protein, 26 aa, synthetic construct [sequence omitted]

SEQ ID NO: 114 - protein, 8 aa, synthetic construct
SSSYLAWY

SEQ ID NO: 115 - protein, 7 aa, synthetic construct
QSVSSSY

SEQ ID NO: 116 - protein, 9 aa, synthetic construct
QQKPGQAPR

SEQ ID NO: 117 - protein, 17 aa, synthetic construct
LAWYQQKPGQAPRLLIY

SEQ ID NO: 118 - protein, 10 aa, synthetic construct
LLIYGASSRA

SEQ ID NO: 119 - protein, 14 aa, Homo sapiens
CARDDWSHYSIKYW

SEQ ID NO: 120 - protein, 33 aa, synthetic construct
AGIPDRFSGSGSGTDFTLTISRLEPEDFAVYYC

SEQ ID NO: 121 - protein, 37 aa, synthetic construct
SSRAAGIPDRFSGSGSGTDFTLTISRLEPEDFAVYYC

SEQ ID NO: 122 - protein, 8 aa, synthetic construct
QQTPLGGW

SEQ ID NO: 123 - protein, 11 aa, synthetic construct
TFGQGTKVEIK

SEQ ID NO: 124 - protein, 124 aa, synthetic construct
QVLLAQSGSEVKNPGSSVRVSCKLSGGTFTTFTFSWLRQAPGQGLEWMGRIIPSLGVADYADKFQGRVTITADKSTSTAYMKVSSLRSEDTAQYYCAKNGGYNYGSYYYYMDVWGQGTTVIVSS

SEQ ID NO: 125 - protein, 122 aa, synthetic construct
QVRLVQSGAEVKKPGASVKVSCQPSGYYFTDYDIHWVRQAPGQGLEWMGWINPNTGATGFAQKFQGRVTMTRDTSIKIGFMQLFSLTSDDTAVYYCARVCCRSTRSRNLDYWGQGTLVTVSS

SEQ ID NO: 126 - protein, 124 aa, synthetic construct
QVLLAQSGSEVKNPGSSVRVSCKLSGGTFTTFTFSWLRQAPGQGLEWMGRIIPSLGVADYADKFQGRVTITADKSTSTAYMKVSSLRSEDTAQYYCARDASSGSYAGRAHFDYWGQGTTVIVSS

SEQ ID NO: 127 - protein, 120 aa, synthetic construct
EVQLVESGGGLVQPGGSLRLSCAGSKFPFSTSWLTWVRQAPGKGLEWLAFIHPDGRITYYADSVRGRFTISRDNARNSVYLQMSSLRDDDTALYYCARHRRAGAHFFDYWGQGTMVTVSS

SEQ ID NO: 128 - protein, 108 aa, synthetic construct
EIVLTQSPGTLSLSPGERATLSCRASQSVSSSYLAWYQQKPGQAPRLLIYGASSRAAGIPDRFSGSGSGTDFTLTISRLEPEDFAVYYCQQTPLGGWTFGQGTKVEIK

SEQ ID NO: 129 - DNA, 372 bp, synthetic construct
  source 1..372: mol_type = other DNA
caggtcctgctggcgcagtctgggtctgaagtgaagaaccctgggtcctccgtgagagtctcctgcaagctttctgggggcaccttcaccaccttcactttcagctggctgcgacaggcccctggacaggggcttgagtggatgggaaggatcatccctagtctaggtgtagcagactatgcagacaaattccaaggcagggtcaccattaccgcggacaaatccacgagcacagcctacatgaaggtcagtagcctgagatctgaggacacggcccaatattactgtgcgaagaatgggggctacaactatggctcctactactactacatggacgtctggggccaagggaccacggtcatcgtctcgtct

SEQ ID NO: 130 - DNA, 366 bp, synthetic construct
  source 1..366: mol_type = other DNA
caggtgcgcctggtgcagtctggggctgaggtaaagaagcctggggcctcagtgaaagtctcctgccaaccttctggatactacttcaccgactacgatatacactgggtgcgacaggcccctggacaagggcttgagtggatgggatggatcaaccctaacactggtgccacaggctttgcacagaagtttcagggcagagtcaccatgaccagggacacgtccatcaaaatagggttcatgcagttgttcagcctgacatctgacgacacggccgtctattactgtgcgagggtttgttgtcgaagcacccgctcccggaatcttgactactggggccagggaaccctggtcaccgtctcctca

SEQ ID NO: 131 - DNA, 372 bp, synthetic construct
  source 1..372: mol_type = other DNA
caggtcctgctggcgcagtctgggtctgaagtgaagaaccctgggtcctccgtgagagtctcctgcaagctttctgggggcaccttcaccaccttcactttcagctggctgcgacaggcccctggacaggggcttgagtggatgggaaggatcatccctagtctaggtgtagcagactatgcagacaaattccaaggcagggtcaccattaccgcggacaaatccacgagcacagcctacatgaaggtcagtagcctgagatctgaggacacggcccaatattactgtgcgagagacgccagtagtgggagctacgccggaagggcccactttgactactggggccaagggaccacggtcatcgtctcgtct

SEQ ID NO: 132 - DNA, 360 bp, synthetic construct
  source 1..360: mol_type = other DNA
gaggtgcagctggtggagtctgggggaggcttggtccagcccggggggtccctgagactctcctgtgcaggctctaaatttccctttagtacctcctggttgacctgggtccgccaggcgccagggaaggggctggagtggctggccttcatacacccagatggaagaattacttattatgcggactctgtgaggggccgattcaccatctccagagacaacgccaggaactcagtgtatcttcaaatgagcagcctgagggacgatgacacggctctttactactgtgcgcgacaccgacgggcaggggctcacttctttgactactggggccaggggacaatggtcaccgtctcttca

SEQ ID NO: 133 - DNA, 324 bp, synthetic construct
  source 1..324: mol_type = other DNA
gaaattgtgttgacgcagtctccaggcaccctgtctttgtctccaggggaaagagccaccctctcctgcagggccagtcagagtgttagcagcagctacttagcctggtaccagcagaaacctggccaggctcccaggctcctcatctatggtgcatccagcagggccgctggcatcccagacaggttcagtggcagtgggtctgggacagacttcactctcaccatcagcagactggagcctgaagattttgcagtgtattactgtcagcagactcctctagggggctggacgttcggtcaagggaccaaggtggaaatcaaa

SEQ ID NO: 134 - protein, 19 aa, Homo sapiens
CARDASSGSYAGRAHFDYW

SEQ ID NO: 135 - protein, 15 aa, Homo sapiens
CARHRRAGAHFFDYW

SEQ ID NO: 136 - protein, 20 aa, Homo sapiens
CARDTSPYISGHDLDAFDIW

SEQ ID NO: 137 - protein, 19 aa, Homo sapiens
CASLGESYYWSENAAFDLW

SEQ ID NO: 138 - protein, 17 aa, Homo sapiens
CAKVEPYSYPRNAYDVW

SEQ ID NO: 139 - protein, 14 aa, Homo sapiens
CARDDWSNYSIKYW

SEQ ID NO: 140 - protein, 19 aa, Homo sapiens
CAKNGGYNYGSYYYYMDVW

SEQ ID NO: 141 - protein, 13 aa, Homo sapiens
CARDPAYGAMDLW

SEQ ID NO: 142 - protein, 17 aa, Homo sapiens
CARVCCRSTRSRNLDYW

SEQ ID NO: 143 - protein, 19 aa, Homo sapiens
CARDASSGSYAGRAHFDYW

SEQ ID NO: 144 - protein, 15 aa, Homo sapiens
CARHRRAGAHFFDYW